European Patent Specification EP 3 149 143 B1, published August 6, 2025. Title: Use of Polypeptide. Applicant: Novozymes A/S. Application -. The sequence listing filed with the application follows.

SEQUENCE LISTING (8 sequences)

SEQ ID NO: 1 - DNA, 910 bp, Aspergillus oryzae
  exon (1)..(242)
  Intron (243)..(308)
  exon (309)..(494)
  Intron (495)..(555)
  exon (556)..(714)
  Intron (715)..(765)
  exon (766)..(907)
  Intron (908)..(910)
atgcagcttactaagtccctcctggtattcgcgctttacatgtttggcactcagcacgttctagctgtgcctgtcaatcccgagcctgatgctacgagcgtcgaaaatgttgcccttaaaacaggcagcggtgatagccagagcgatcccatcaaggcggacttggaggtcaaaggccaaagtgctttgcctttcgacgtcgactgctgggctatcctgtgcaagggcgccccgaatgtcctgtatgtcttcctttattgaagctcttgatgtggcttgtatgtttgactaatatatcgcacccttaggcagcgcgtgaatgaaaagacgaaaaatagtaatcgcgatcggagcggtgcgaacaaagggcctttcaaagatcctcagaaatggggcatcaaagcccttccacctaagaatccatcctggagcgcacaagacttcaaatcacccgaagaatacgcatttgcgtcttcccttcaaggcggaaccaagtatgctaagatcatcactgcttcaatcaatgtgttgttagctgactccgatgtgaccaagtgccatcctagcgcccgtcaacctcgcttctcagaactcccaaggcggcgtcttgaacggtttctactcggcgaacaaagtagcacaatttgatcctagcaagccccaacagacaaagggaacatggtttcagatcactaagttcacaggtgcagctgggtaagaacttccagtaccatggtcatatgcaatttactaagaaaatactagtccttactgcaaggctctggggagtaatgataagagtgtgtgcgataagaacaagaatattgcaggggactggggcttcgacccggcgaaatgggcatatcagtatgatgagaagaataacaagttcaactatgttggtaagtaa

SEQ ID NO: 2 - protein, 243 aa, Aspergillus oryzae
  SIGNAL (1)..(22)
  PROPEP (23)..(37)
  PEPTIDE (38)..(243)
MQLTKSLLVFALYMFGTQHVLAVPVNPEPDATSVENVALKTGSGDSQSDPIKADLEVKGQSALPFDVDCWAILCKGAPNVLQRVNEKTKNSNRDRSGANKGPFKDPQKWGIKALPPKNPSWSAQDFKSPEEYAFASSLQGGTNAILAPVNLASQNSQGGVLNGFYSANKVAQFDPSKPQQTKGTWFQITKFTGAAGPYCKALGSNDKSVCDKNKNIAGDWGFDPAKWAYQYDEKNNKFNYVGK

SEQ ID NO: 3 - protein, 204 aa, Aspergillus oryzae
  PEPTIDE (1)..(204)
KTGSGDSQSDPIKADLEVKGQSALPFDVDCWAILCKGAPNVLQRVNEKTKNSNRDRSGANKGPFKDPQKWGIKALPPKNPSWSAQDFKSPEEYAFASSLQGGTNAILAPVNLASQNSQGGVLNGFYSANKVAQFDPSKPQQTKGTWFQITKFTGAAGPYCKALGSNDKSVCDKNKNIAGDWGFDPAKWAYQYDEKNNKFNYVGK

SEQ ID NO: 4 - DNA, 868 bp, Trichoderma harzianum
  exon (1)..(75)
  Intron (76)..(154)
  exon (155)..(288)
  Intron (289)..(362)
  exon (363)..(519)
  Intron (520)..(615)
  exon (616)..(867)
atgaagctgtccatctctgtcgctcttacttcggccatcgcggttctcgccgccccggctcctatgcctacaccggtatgtagcatcaatgcaacatgacataacttgtatctcgactatatatcagactggctaatgcttcaactcattacagcccggtattcccacggaaagcagcgccagaacccaacttgccggcctgactgttgccgttgctggctctggaactggttactcccgcgacctgtttcccacttgggatgccatctctggtaactgcaacgctcggtatgataacatcctaggacctttcaagcttcggaaatacaacacaaaggctaacaaagtggatgtgcaaatagcgaatatgtgttgaagcgagatggtgaaggtgtccaagtcaacaatgcttgtgaatctcagtccggcacctggatcagatccttatgacaacgccagtttcacaaatgcatccagcttggatattgaccacatggtgcctctaaagaatgcctggatcgtgagttttctcctttttcactgcgtatctccgttccctacctttttgcgatactatatcatgccacatcactaatatggacaaatttctcgccagtccggtgcctcaagctggaccacagcccaacgtgaagccctcgccaacgacgtctcccgtccccaactctgggccgtctccgcaagcgcaaaccgctccaagggcgaccgcagcccagaccagtggaagcctcctctgaccagcttctactgcacctacgccaagtcgtggatcgatgtcaagagcttctataagctgacaatcaccagtgccgagaagacagctctgagcagcatgttagatacttgctag

SEQ ID NO: 5 - protein, 205 aa, Trichoderma harzianum
  SIGNAL (1)..(17)
  PEPTIDE (18)..(205)
MKLSISVALTSAIAVLAAPAPMPTPPGIPTESSARTQLAGLTVAVAGSGTGYSRDLFPTWDAISGNCNAREYVLKRDGEGVQVNNACESQSGTWISPYDNASFTNASSLDIDHMVPLKNAWISGASSWTTAQREALANDVSRPQLWAVSASANRSKGDRSPDQWKPPLTSFYCTYAKSWIDVKSFYKLTITSAEKTALSSMLDTC

SEQ ID NO: 6 - protein, 136 aa, Bacillus subtilis
  SIGNAL (1)..(26)
  PEPTIDE (27)..(136)
MKKWMAGLFLAAAVLLCLMVPQQIQGASSYDKVLYFPLSRYPETGSHIRDAIAEGHPDICTIDRDGADKRREESLKGIPTKPGYDRDEWPMAVCEEGGAGADVRYVTPSDNRGAGSWVGNQMSSYPDGTRVLFIVQ

SEQ ID NO: 7 - protein, 142 aa, Bacillus licheniformis
  SIGNAL (1)..(33)
  PEPTIDE (34)..(136)
MIKKWAVHLLFSALVLLGLSGGAAYSPQHAEGAARYDDILYFPASRYPETGAHISDAIKAGHSDVCTIERSGADKRRQESLKGIPTKPGFDRDEWPMAMCEEGGKGASVRYVSSSDNRGAGSWVGNRLSGFADGTRILFIVQ

SEQ ID NO: 8 - protein, 206 aa, Aspergillus oryzae
ALKTGSGDSQSDPIKADLEVKGQSALPFDVDCWAILCKGAPNVLQRVNEKTKNSNRDRSGANKGPFKDPQKWGIKALPPKNPSWSAQDFKSPEEYAFASSLQGGTNAILAPVNLASQNSQGGVLNGFYSANKVAQFDPSKPQQTKGTWFQITKFTGAAGPYCKALGSNDKSVCDKNKNIAGDWGFDPAKWAYQYDEKNNKFNYVGK